European Patent Specification EP 3 677 285 B1, published December 13, 2023. Title: TARGETING PEPTIDES AND METHODS OF USE. Applicant: Case Western Reserve University. The sequence listing filed with the application follows.

SEQUENCE LISTING (41 sequences)

SEQ ID NO: 1 - protein, 7 aa, Homo sapiens
TVRTSAD

SEQ ID NO: 2 - protein, 7 aa, Homo sapiens
NWGDRIL

SEQ ID NO: 3 - protein, 7 aa, Homo sapiens
NWGKPIK

SEQ ID NO: 4 - protein, 7 aa, Homo sapiens
SGVKSAF

SEQ ID NO: 5 - protein, 7 aa, Homo sapiens
GVKSYNE

SEQ ID NO: 6 - protein, 7 aa, Homo sapiens
IGKTNTL

SEQ ID NO: 7 - protein, 7 aa, Homo sapiens
IGNSNTL

SEQ ID NO: 8 - protein, 7 aa, Homo sapiens
IGNTIPV

SEQ ID NO: 9 - protein, 7 aa, Homo sapiens
LYANSPF

SEQ ID NO: 10 - protein, 9 aa, Homo sapiens
CTVRTSADC

SEQ ID NO: 11 - protein, 9 aa, Homo sapiens
CNWGDRILC

SEQ ID NO: 12 - protein, 9 aa, Homo sapiens
CNWGKPIKC

SEQ ID NO: 13 - protein, 9 aa, Homo sapiens
CSGVKSAFC

SEQ ID NO: 14 - protein, 9 aa, Homo sapiens
CGVKSYNEC

SEQ ID NO: 15 - protein, 9 aa, Homo sapiens
CIGKTNTLC

SEQ ID NO: 16 - protein, 9 aa, Homo sapiens
CIGNSNTLC

SEQ ID NO: 17 - protein, 9 aa, Homo sapiens
CIGNTIPVC

SEQ ID NO: 18 - protein, 9 aa, Homo sapiens
CLYANSPFC

SEQ ID NO: 19 - protein, 7 aa, Homo sapiens
WNYPFRL

SEQ ID NO: 20 - protein, 7 aa, Homo sapiens
SNTSYVN

SEQ ID NO: 21 - protein, 7 aa, Homo sapiens
SFSYTSG

SEQ ID NO: 22 - protein, 7 aa, Homo sapiens
WSPAPMS

SEQ ID NO: 23 - protein, 7 aa, Homo sapiens
TREHPAQ

SEQ ID NO: 24 - protein, 7 aa, Homo sapiens
ARIIDNA

SEQ ID NO: 25 - protein, 9 aa, Homo sapiens
CWNYPFRLC

SEQ ID NO: 26 - protein, 9 aa, Homo sapiens
CSNTSYVNC

SEQ ID NO: 27 - protein, 9 aa, Homo sapiens
CSFSYTSGC

SEQ ID NO: 28 - protein, 9 aa, Homo sapiens
CWSPAPMSC

SEQ ID NO: 29 - protein, 9 aa, Homo sapiens
CTREHPAQC

SEQ ID NO: 30 - protein, 9 aa, Homo sapiens
CARIIDNAC

SEQ ID NO: 31 - DNA, 19 bp, Homo sapiens
gcagcccacagtggagtat

SEQ ID NO: 32 - DNA, 20 bp, Homo sapiens
ggagcaaggttgatttcttt

SEQ ID NO: 33 - DNA, 19 bp, Homo sapiens
gcagcccacagtggagtat

SEQ ID NO: 34 - DNA, 20 bp, Homo sapiens
ggagcaaggttgatttcttt

SEQ ID NO: 35 - DNA, 20 bp, Homo sapiens
acccagaagactgtggatgg

SEQ ID NO: 36 - DNA, 20 bp, Homo sapiens
tctagacggcaggtcaggtc

SEQ ID NO: 37 - DNA, 20 bp, Homo sapiens
tgcccagaaaatgaaaaagg

SEQ ID NO: 38 - DNA, 20 bp, Homo sapiens
gtgtatgtggcaatgcgttc

SEQ ID NO: 39 - DNA, 20 bp, Homo sapiens
acagtggccacctacaaagg

SEQ ID NO: 40 - DNA, 20 bp, Homo sapiens
ccgagatggggttgataatg

SEQ ID NO: 41 - protein, 9 aa, Homo sapiens
TVRTSADCC